European Patent Specification EP 3 436 606 B1, published February 22, 2023. Title: PLASMA DERIVED CELL-FREE MITOCHONDRIAL DEOXYRIBONUCLEIC ACID. Applicant: UTI Limited Partnership UTI Limited Partnership. The sequence listing filed with the application follows.

SEQUENCE LISTING (4 sequences)

SEQ ID NO: 1 - DNA, 20 bp, Artificial Sequence
  Forward Primer "MTL1"
aaagcacataccaaggccac

SEQ ID NO: 2 - DNA, 22 bp, Artificial Sequence
  Reverse Primer "MTL1"
ggttctgtgggcaaatttaaag

SEQ ID NO: 3 - DNA, 22 bp, Artificial Sequence
  Forward Primer "MTL2"
tgaggccaaatatcattctgag

SEQ ID NO: 4 - DNA, 20 bp, Artificial Sequence
  Reverse Primer "MTL2"
aatgttgagccgtagatgcc